European Patent Application EP 4 257 692 A1, published October 11, 2023. Title: Recombinant Microorganism Having Enhanced Ability to Produce Recombinant Silk Protein and Method for Producing High Molecular Weight Recombinant Silk Protein Using The Same. Applicant: KAIST. The sequence listing filed with the application follows.

SEQUENCE LISTING (87 sequences)

SEQ ID NO: 1 - protein, 35 aa, Artificial Sequence
  Artificial sequence
SGRGGLGGQGAGMAAAAAMGGAGQGGYGGLGSQGT

SEQ ID NO: 2 - protein, 5 aa, Artificial Sequence
  Artificial sequence
GPGQQ

SEQ ID NO: 3 - protein, 5 aa, Artificial Sequence
  Artificial sequence
GPGGY

SEQ ID NO: 4 - protein, 7 aa, Artificial Sequence
  Artificial sequence
GGYGPGS

SEQ ID NO: 5 - protein, 5 aa, Artificial Sequence
  Artificial sequence
GVGVP

SEQ ID NO: 6 - protein, 4 aa, Artificial Sequence
  Artificial sequence
VPGG

SEQ ID NO: 7 - protein, 6 aa, Artificial Sequence
  Artificial sequence
APGVGV

SEQ ID NO: 8 - protein, 6 aa, Artificial Sequence
  Artificial sequence
GAGAGS

SEQ ID NO: 9 - protein, 5 aa, Artificial Sequence
  Artificial sequence
GPGGG

SEQ ID NO: 10 - protein, 5 aa, Artificial Sequence
  Artificial sequence
  misc_feature (5)..(5): Xaa can be any naturally occurring amino acid
GPGGX

SEQ ID NO: 11 - protein, 15 aa, Artificial Sequence
  Artificial sequence
GAPGAPGSQGAPGLQ

SEQ ID NO: 12 - protein, 15 aa, Artificial Sequence
  Artificial sequence
GAPGTPGPQGLPGSP

SEQ ID NO: 13 - DNA, 49 bp, Artificial Sequence
  Artificial sequence
taacaccgtgcgtgttgactattttacctctggcggtgataatggttgc

SEQ ID NO: 14 - DNA, 79 bp, Artificial Sequence
  Artificial sequence
tttctgttgggccattgcattgccactgattttccaacatataaaaagacaagcccgaacagtcgtccgggcttttttt

SEQ ID NO: 15 - DNA, 129 bp, Artificial Sequence
  Artificial sequence
ccaggcatcaaataaaacgaaaggctcagtcgaaagactgggcctttcgttttatctgttgtttgtcggtgaacgctctctactagagtcacactggctcaccttcgggtgggcctttctgcgtttata

SEQ ID NO: 16 - DNA, 18 bp, Artificial Sequence
  Artificial sequence
atgtccaaaatcgtaaaa

SEQ ID NO: 17 - DNA, 24 bp, Artificial Sequence
  Artificial sequence
atgatttcaggcattttagcatcc

SEQ ID NO: 18 - DNA, 24 bp, Artificial Sequence
  Artificial sequence
atgaaaaccgcttacattgccaaa

SEQ ID NO: 19 - DNA, 20 bp, Artificial Sequence
  Artificial sequence
gtgaacaaaatattttcctc

SEQ ID NO: 20 - DNA, 24 bp, Artificial Sequence
  Artificial sequence
atgagtcaggcgctaaaaaattta

SEQ ID NO: 21 - DNA, 24 bp, Artificial Sequence
  Artificial sequence
atgaaaaaattgatcaatgatgtg

SEQ ID NO: 22 - DNA, 24 bp, Artificial Sequence
  Artificial sequence
atgacggaaaacattcataagcat

SEQ ID NO: 23 - DNA, 24 bp, Artificial Sequence
  Artificial sequence
atgcgcgttaacaatggtttgacc

SEQ ID NO: 24 - DNA, 24 bp, Artificial Sequence
  Artificial sequence
atgacgttattaggcactgcgctg

SEQ ID NO: 25 - DNA, 24 bp, Artificial Sequence
  Artificial sequence
atgtccaaaatcgtaaaaatcatc

SEQ ID NO: 26 - DNA, 23 bp, Artificial Sequence
  Artificial sequence
atgtccaaaatcgtaaaaatcat

SEQ ID NO: 27 - DNA, 22 bp, Artificial Sequence
  Artificial sequence
atgtccaaaatcgtaaaaatca

SEQ ID NO: 28 - DNA, 21 bp, Artificial Sequence
  Artificial sequence
atgtccaaaatcgtaaaaatc

SEQ ID NO: 29 - DNA, 20 bp, Artificial Sequence
  Artificial sequence
atgtccaaaatcgtaaaaat

SEQ ID NO: 30 - DNA, 19 bp, Artificial Sequence
  Artificial sequence
atgtccaaaatcgtaaaaa

SEQ ID NO: 31 - DNA, 17 bp, Artificial Sequence
  Artificial sequence
atgtccaaaatcgtaaa

SEQ ID NO: 32 - DNA, 16 bp, Artificial Sequence
  Artificial sequence
atgtccaaaatcgtaa

SEQ ID NO: 33 - DNA, 15 bp, Artificial Sequence
  Artificial sequence
atgtccaaaatcgta

SEQ ID NO: 34 - DNA, 28 bp, Artificial Sequence
  Artificial sequence
gcaaccattatcaccgccagaggtaaaa

SEQ ID NO: 35 - DNA, 45 bp, Artificial Sequence
  Artificial sequence
gatgatttttacgattttggacattttctgttgggccattgcatt

SEQ ID NO: 36 - DNA, 44 bp, Artificial Sequence
  Artificial sequence
atgatttttacgattttggacattttctgttgggccattgcatt

SEQ ID NO: 37 - DNA, 43 bp, Artificial Sequence
  Artificial sequence
tgatttttacgattttggacattttctgttgggccattgcatt

SEQ ID NO: 38 - DNA, 42 bp, Artificial Sequence
  Artificial sequence
gatttttacgattttggacattttctgttgggccattgcatt

SEQ ID NO: 39 - DNA, 41 bp, Artificial Sequence
  Artificial sequence
atttttacgattttggacattttctgttgggccattgcatt

SEQ ID NO: 40 - DNA, 40 bp, Artificial Sequence
  Artificial sequence
tttttacgattttggacattttctgttgggccattgcatt

SEQ ID NO: 41 - DNA, 39 bp, Artificial Sequence
  Artificial sequence
ttttacgattttggacattttctgttgggccattgcatt

SEQ ID NO: 42 - DNA, 38 bp, Artificial Sequence
  Artificial sequence
tttacgattttggacattttctgttgggccattgcatt

SEQ ID NO: 43 - DNA, 37 bp, Artificial Sequence
  Artificial sequence
ttacgattttggacattttctgttgggccattgcatt

SEQ ID NO: 44 - DNA, 37 bp, Artificial Sequence; identical to SEQ ID NO: 43
  Artificial sequence

SEQ ID NO: 45 - DNA, 24 bp, Artificial Sequence
  Artificial sequence
gtgaacaaaatattttcctcacat

SEQ ID NO: 46 - DNA, 23 bp, Artificial Sequence
  Artificial sequence
gtgaacaaaatattttcctcaca

SEQ ID NO: 47 - DNA, 22 bp, Artificial Sequence
  Artificial sequence
gtgaacaaaatattttcctcac

SEQ ID NO: 48 - DNA, 21 bp, Artificial Sequence
  Artificial sequence
gtgaacaaaatattttcctca

SEQ ID NO: 49 - DNA, 19 bp, Artificial Sequence
  Artificial sequence
gtgaacaaaatattttcct

SEQ ID NO: 50 - DNA, 18 bp, Artificial Sequence
  Artificial sequence
gtgaacaaaatattttcc

SEQ ID NO: 51 - DNA, 17 bp, Artificial Sequence
  Artificial sequence
gtgaacaaaatattttc

SEQ ID NO: 52 - DNA, 16 bp, Artificial Sequence
  Artificial sequence
gtgaacaaaatatttt

SEQ ID NO: 53 - DNA, 15 bp, Artificial Sequence
  Artificial sequence
gtgaacaaaatattt

SEQ ID NO: 54 - DNA, 28 bp, Artificial Sequence
  Artificial sequence
gcaaccattatcaccgccagaggtaaaa

SEQ ID NO: 55 - DNA, 41 bp, Artificial Sequence
  Artificial sequence
acgccaaaaattgaacacattttctgttgggccattgcatt

SEQ ID NO: 56 - DNA, 41 bp, Artificial Sequence
  Artificial sequence
gcaatgtaagcggttttcattttctgttgggccattgcatt

SEQ ID NO: 57 - DNA, 41 bp, Artificial Sequence
  Artificial sequence
aaaccattgttaacgcgcattttctgttgggccattgcatt

SEQ ID NO: 58 - DNA, 41 bp, Artificial Sequence
  Artificial sequence
agtactaacttactcgacattttctgttgggccattgcatt

SEQ ID NO: 59 - DNA, 41 bp, Artificial Sequence
  Artificial sequence
agcataataatacgggacactttctgttgggccattgcatt

SEQ ID NO: 60 - DNA, 41 bp, Artificial Sequence
  Artificial sequence
gctaaaatgcctgaaatcattttctgttgggccattgcatt

SEQ ID NO: 61 - DNA, 41 bp, Artificial Sequence
  Artificial sequence
cgaaaaaagctaaaaagcattttctgttgggccattgcatt

SEQ ID NO: 62 - DNA, 41 bp, Artificial Sequence
  Artificial sequence
ccgatctgttgcttggacattttctgttgggccattgcatt

SEQ ID NO: 63 - DNA, 41 bp, Artificial Sequence
  Artificial sequence
aaaagcttcatatcaggcactttctgttgggccattgcatt

SEQ ID NO: 64 - DNA, 41 bp, Artificial Sequence
  Artificial sequence
acaaccggaaattcattcattttctgttgggccattgcatt

SEQ ID NO: 65 - DNA, 41 bp, Artificial Sequence
  Artificial sequence
ttttttagcgcctgactcattttctgttgggccattgcatt

SEQ ID NO: 66 - DNA, 41 bp, Artificial Sequence
  Artificial sequence
cgttcttcgatagtgctcattttctgttgggccattgcatt

SEQ ID NO: 67 - DNA, 41 bp, Artificial Sequence
  Artificial sequence
tcattttgcgcttcagccattttctgttgggccattgcatt

SEQ ID NO: 68 - DNA, 41 bp, Artificial Sequence
  Artificial sequence
actatgaccaggtttaccattttctgttgggccattgcatt

SEQ ID NO: 69 - DNA, 41 bp, Artificial Sequence
  Artificial sequence
tcattgatcaattttttcattttctgttgggccattgcatt

SEQ ID NO: 70 - DNA, 41 bp, Artificial Sequence
  Artificial sequence
tgagttctgctcagtgacattttctgttgggccattgcatt

SEQ ID NO: 71 - DNA, 41 bp, Artificial Sequence
  Artificial sequence
ttgttaaaagcgccactcattttctgttgggccattgcatt

SEQ ID NO: 72 - DNA, 41 bp, Artificial Sequence
  Artificial sequence
gtatccagatacagttccattttctgttgggccattgcatt

SEQ ID NO: 73 - DNA, 41 bp, Artificial Sequence
  Artificial sequence
gtgtccagatacagttccattttctgttgggccattgcatt

SEQ ID NO: 74 - DNA, 41 bp, Artificial Sequence
  Artificial sequence
ttatgaatgttttccgtcattttctgttgggccattgcatt

SEQ ID NO: 75 - DNA, 41 bp, Artificial Sequence
  Artificial sequence
gtaacttcttgctggaacattttctgttgggccattgcatt

SEQ ID NO: 76 - DNA, 41 bp, Artificial Sequence
  Artificial sequence
gcagtgcctaataacgtcattttctgttgggccattgcatt

SEQ ID NO: 77 - DNA, 41 bp, Artificial Sequence
  Artificial sequence
cgaacgaaggggtagtacattttctgttgggccattgcatt

SEQ ID NO: 78 - DNA, 45 bp, Artificial Sequence
  Artificial sequence
atgtgaggaaaatattttgttcactttctgttgggccattgcatt

SEQ ID NO: 79 - DNA, 44 bp, Artificial Sequence
  Artificial sequence
tgtgaggaaaatattttgttcactttctgttgggccattgcatt

SEQ ID NO: 80 - DNA, 43 bp, Artificial Sequence
  Artificial sequence
gtgaggaaaatattttgttcactttctgttgggccattgcatt

SEQ ID NO: 81 - DNA, 42 bp, Artificial Sequence
  Artificial sequence
tgaggaaaatattttgttcactttctgttgggccattgcatt

SEQ ID NO: 82 - DNA, 41 bp, Artificial Sequence
  Artificial sequence
gaggaaaatattttgttcactttctgttgggccattgcatt

SEQ ID NO: 83 - DNA, 40 bp, Artificial Sequence
  Artificial sequence
aggaaaatattttgttcactttctgttgggccattgcatt

SEQ ID NO: 84 - DNA, 39 bp, Artificial Sequence
  Artificial sequence
ggaaaatattttgttcactttctgttgggccattgcatt

SEQ ID NO: 85 - DNA, 38 bp, Artificial Sequence
  Artificial sequence
gaaaatattttgttcactttctgttgggccattgcatt

SEQ ID NO: 86 - DNA, 37 bp, Artificial Sequence
  Artificial sequence
aaaatattttgttcactttctgttgggccattgcatt

SEQ ID NO: 87 - DNA, 36 bp, Artificial Sequence
  Artificial sequence
aaatattttgttcactttctgttgggccattgcatt